European Patent Application EP 4 141 022 A1, published March 1, 2023. Title: Feline calicivirus vaccine. Applicant: Intervet International B.V. The sequence listing filed with the application follows.

SEQUENCE LISTING (66 sequences)

SEQ ID NO: 1 - DNA, 50 bp, Feline calicivirus
catggtacctaatacgactcactatagggtaaaagaaatttgagacaatg

SEQ ID NO: 2 - DNA, 49 bp, Feline calicivirus
tcgaccaccggtgattaattttttttttttttttttttttttccctggg

SEQ ID NO: 3 - DNA, 67 bp, Feline calicivirus
tacctaatacgactcactatagggtaaaagaaatttgagacaatgtctcaaactctgagcttcgtgc

SEQ ID NO: 4 - DNA, 48 bp, Feline calicivirus
ttttttttttttttttttttttttccctggggttaggcgcaggtgcgg

SEQ ID NO: 5 - DNA, 44 bp, Feline calicivirus
gtaaaagaaatttgagacaatgtctcaaactctgagcttcgtgc

SEQ ID NO: 6 - DNA, 53 bp, Feline calicivirus
atagtatttaagcacgttagcgcaggttgagcacatgctcaaacttcgaacac

SEQ ID NO: 7 - DNA, 52 bp, Feline calicivirus
gagtggcatgaccgccctacactgtgatgtgttcgaagtttgagcatgtgct

SEQ ID NO: 8 - DNA, 36 bp, Feline calicivirus
ttttttttttttccctggggttaggcgcaggtgcgg

SEQ ID NO: 9 - DNA, 36 bp, Feline calicivirus
cttggtaccgagctgtaaaagaaatttgagacaatg

SEQ ID NO: 10 - DNA, 18 bp, Feline calicivirus
tgagctgttctttgcaca

SEQ ID NO: 11 - DNA, 21 bp, Feline calicivirus
ctccttgaaagagttggtgtg

SEQ ID NO: 12 - DNA, 20 bp, Feline calicivirus
ctatggtgcattcggtgatg

SEQ ID NO: 13 - DNA, 20 bp, Feline calicivirus
gcgacaactcttgtatcagg

SEQ ID NO: 14 - DNA, 20 bp, Feline calicivirus
gacatgcttgagaacaaggg

SEQ ID NO: 15 - DNA, 16 bp, Feline calicivirus
gaactacccgccaatc

SEQ ID NO: 16 - DNA, 15 bp, Feline calicivirus
gagcccaggccaaat

SEQ ID NO: 17 - DNA, 31 bp, Feline calicivirus
gatcggtcgacgagctcttctctctcttagg

SEQ ID NO: 18 - DNA, 20 bp, Feline calicivirus
gtatgacgtaacaaagcctg

SEQ ID NO: 19 - DNA, 20 bp, Feline calicivirus
ggaaattggcaacccaaggc

SEQ ID NO: 20 - DNA, 20 bp, Feline calicivirus
gctgtaaaagtgtcctctgg

SEQ ID NO: 21 - DNA, 19 bp, Feline calicivirus
cactgtgatgtgttcgaag

SEQ ID NO: 22 - DNA, 18 bp, Feline calicivirus
tatttaagcacgttagcg

SEQ ID NO: 23 - DNA, 20 bp, Feline calicivirus
catcttatgtcagatactga

SEQ ID NO: 24 - DNA, 20 bp, Feline calicivirus
ttttcttttgttggtgtctc

SEQ ID NO: 25 - DNA, 34 bp, Feline calicivirus
cgagcggccgccactgtgccctggggttaggcgc

SEQ ID NO: 26 - DNA, 18 bp, Feline calicivirus
gggagatgagaagcttcg

SEQ ID NO: 27 - DNA, 19 bp, Feline calicivirus
gcccaaactatgaaacaag

SEQ ID NO: 28 - DNA, 20 bp, Feline calicivirus
aacgccattggatctgtaac

SEQ ID NO: 29 - DNA, 20 bp, Feline calicivirus
attgaaccaatcgatcctga

SEQ ID NO: 30 - DNA, 20 bp, Feline calicivirus
tcaggatcgattggttcaat

SEQ ID NO: 31 - DNA, 32 bp, Feline calicivirus
ttccaggtacctccggaaggagttctgggtag

SEQ ID NO: 32 - DNA, 53 bp, Feline calicivirus
agagctctctggctaacgtaaaagaaatttgagacaatgtctcaaactctgag

SEQ ID NO: 33 - DNA, 34 bp, Feline calicivirus
ggcaactagaaggcacagccctggggttaggcgc

SEQ ID NO: 34 - protein, 668 aa, Feline calicivirus
MCSTCANVLKYYDWDPHFKLVIDPNKFLSVGFCDNPLMCCYPELLPEFGTVWDCDQSPLQIYLESILGDDEWSSTYEAIDPVVPPMHWDKMGKIFQPHPGMLMHHIIGEVAKGWDPNLPLFRLEADDGSVTTPEQGTMVGGVIAEPSAQMSTAADMASGKSVDSEWEAFFSFHTSVNWSTSETQGKILFKQSLGPLLNPYLEHISKLYVAWSGSIEVRFSISGSGVFGGKLAAIVVPPGVDPVQSTSMLQYPHVLFDARQVEPVIFSIPDLRNSLYHLMSDTDTTSLVIMVYNDLINPYANDSNSSGCIVTVETKPGIDFKFHLLKPPGSMLTHGSIPSDLIPKSSSLWIGNRHWTDITDFVIRPFVFQANRHFDFNQETAGWSTPRFRPLAVTVSQSKGAKLGNGIATDYIVPGIPDGWPDTTIPTKLTPTGDYAITSSDGNDIETKLEYENADVIKNNTNFRSMYICGSLQRAWGDKKISNTGFITTGVISDNSISPSNTIDQSKIVVYQDNHVNSEVQTSDITLAILGYTGIGEEAIGANRDSVVRISVLPETGARGGNHPIFYKNSMKLGYVISSIDVFNSQILHTSRQLSLNNYLLPPDSFAVYRIIDSNGSWFDIGIDSDGFSFVGVSSFPKLEFPLSASYMGIQLAKIRLASNIRSSMTKL

SEQ ID NO: 35 - protein, 671 aa, Feline calicivirus
MCSTCANVLKYYDWDPHFKLVINPNNFLSVGFCSNPLMCCYPELLPEFGTVWDCDRSPLEIYLESILGDDEWASTFDAVDPVVPPMHWGAAGKIFQPHPGVLMHHLIGKVAAGWDPDLPLIRLEADDGSITAPEQGTMVGGVIAEPSAQMSTAADMATGKSVDSEWEAFFSFHTSVNWSTSETQGKILFKQSLGPLLNPYLEHLAKLYVAWSGSIEVRFSISGSGVFGGKLAAIVVPPGVDPVQSTSMLQYPHVLFDARQVEPVIFCLPDLRSTLYHLMSDTDTTSLVIMVYNDLINPYANDANSSGCIVTVETKPGPDFKFHLLKPPGSMLTHGSIPSDLIPKTSSLWIGNRYWSDITDFVIRPFVFQANRHFDFNQETAGWSTPRFRPISVTITEQNGAKLGIGVATDYIVPGIPDGWPDTTIPGELIPAGDYAITNGTGNDITTATGYDTADIIKNNTNFRGMYICGSLQRAWGDKKISNTAFITTATLDGDNNNKINPCNTIDQSKIVVFQDNHVGKKAQTSDDTLALLGYTGIGEQAIGSDRDRVVRISTLPETGARGGNHPIFYKNSIKLGYVIRSIDVFNSQILHTSRQLSLNHYLLPPDSFAVYRIIDSNGSWFDIGIDSDGFSFVGVSGFGKLEFPLSASYMGIQLAKIRLASNIRSPMTKL

SEQ ID NO: 36 - protein, 668 aa, Feline calicivirus
MCSTCANVLKYYDWDPHFKLIINPNKFLSVGFCDNPLMCCYPELLPEFGTVWNCNQSPLQIYLESILGDDEWVSTYEAIDPVVPPMHWNEAGKLFQPHPGILMHHIIGEVAKAWDPNLPLFRLEADDGSITTPEQGTPVGGVIAEPSAQMSAAADMATGKSVDSEWEAFFSFHTSVNWSTSETQGKILFKQSLGPLLNPYLSHLAKLYVAWSGSIEVRFSISGSGVFGGKLAAIIVPPGIEPVQSTSMLQYPHVLFDARQVEPVIFTIPDLRSNLYHLMSDTDTTSLVIMIYNDLINPYANDSNSSGCIVTVETKPGADFKFHLLKPPGSMLTHGSIPSDLIPKSSSLWIGNRHWTDITEFVVRPFVFQANRHFDFNQETAGWSTPRFRPITVTVSEKGGSKLGIGVATDSIVPGIPDGWPDTSISDTLIPSGDYAITSGNGNDIITGADYDSADVIKNNTNFRSMYICGSLQRAWGDKKVSETAFITTAVRNENSISPSNVIDATKLIVYQDAHVETDVQTSDVTLAILGYTGIGEEAIGLDRDKVVRISILPETGTRGGNHPIFYKNSIKLGYVIRSIDVMNSQILHTSRQLSLNNYSLPPDSFAVYRIIDSAGSWFDIGIDSDGFSFVGISNVGKLIFPLSASYMGIQLAKIRLASNIRSAMTKL

SEQ ID NO: 37 - protein, 669 aa, Feline calicivirus
MCSTCANVLKYYDWDPHFRLTINPNKFLSVGFCDNPLMCCYPELLPEFGTVWDCNQSPLEIYLESILGDDEWASTYEAIDPVVPPMHWDCAGKIFQPHPGVLMHHLISEVAKGWDPNLPSFRLEADDGSITTPEQGTPVGGVIAEPSAQMSTAADMASGKSVDSEWGKAFFSFHTSVNWSTSETQGKILFKQSLGPLLNPYLEHLAKLYVAWSGSVEVRFSISGSGVFGGKLAAIVVPPGVDPVQSTSMLQYPHVLFDARQVEPVIFTIPDLRNSLYHLMSDTDTTSLVIMVYNDLINPYASDSNSSGCIVTVETKPGPDFKFHLLKPPGSMLTHGSVPSDLIPKSSSLWIGNRYWSDITDFVIRPFVFQANRHFDFNQETAGWSTPRFRPLTITISVEGGAKLGTGVATDYIVPGIPDGWPDTTIPEKLTPAGDYAITDGNGSDIVTAAKYDTADVIKNNTNFKGMYICGSLQRAWGDKKISNTAFITTGTVENNSIEPSNTIDATKLAVFQDTHVGHEVQTSDDTLALLGYTGIGEQAIGSDRDRVVRISVLPETGARGGNHPIFYKNSIKLGYVIRSIDVFNSQILHTSRQLSLNHYLLPPDSFAVYRIIDSNGSWFDIGIDSDGFSFVGVSSITKLEFPLTASYMGIQLAKIRLASNIRGQMTKI

SEQ ID NO: 38 - protein, 669 aa, Feline calicivirus
MCSTCANVLKYYDWDPHFRLTINPNKFLSVGFCDNPLMCCYPELLPEFGTVWDCDQSPLEIYLESILGDDEWASTYEAIDPVVPPMHWDCAGKIFQPHPGVLMHHLISEVAKGWDPNLPSFRLEADDGSITTPEQGTPVGGVIAEPSAQMSTAADMASGKSVDSEWGKAFFSFHTSVNWSTSETQGKILFKQSLGPLLNPYLEHLAKLYVAWSGSVEVRFSISGSGVFGGKLAAIVVPPGVDPVQSTSMLQYPHVLFDARQVEPVIFTIPDLRNSLYHLMSDTDTTSLVIMVYNDLINPYASDSNSSGCIVTVETKPGPDFKFHLLKPPGSMLTHGSVPSDLIPKSSSLWIGICLWRGITDFVIRPFVFQVNRHFDFNQETAGWSTPRFRPLTITISVKEGANSELGVATDYIVPGIPDGWPDTTIPEKLTPAGDYAITDSSGSDITTAAKYDAADVIENNTNFKGMYICGSLQRAWGDKKISNTAFITTGTVEDNFIEPSNTIDATKLAVFQDTHVGREVQTSDDTLALLGYTGIGEQAIGSDRDRVVRISVLPETGARGGNHPIFYKNSIKLGYVVRSIDVFNSQILHTSRQLSLNHYLLPPDSFAVYRIIDSNGSWFDIGIDSDGFSFVGVSSITKLEFPLTASYMGIQLAKIRLASNIRSQMTKI

SEQ ID NO: 39 - protein, 668 aa, Feline calicivirus
MCSTCANVLKYYNWDPHFKLVINPNKFLPIGFCDNPLMCCYPELLPEFGTVWDCDQSPLQIYLESILGDDEWSSTYEAIDPVVPPMHWDKAGKIFQPHPGVLMHYIIGEVAKAWDPNLPLFRLEADDGSITTPEQGTVVGGVIAEPSSQMSTAADMASGKSVDSEWEAFFSFHTSVNWSTSETQGKILFKQSLGPLLNPYLEHLSKLYVAWSGSVEVRFSISGSGVFGGKLAAIVVPPGVDPIQSTSMLQYPHVLFDARQVEPVIFTIPDLRSTLYHLMSDTDTTSLVVMVYNDLINPYANDSNSSGCIVTVETKPGSDFKFHLLKPPGSVLTHGSVPSDLIPRTSSLWIGNRFWTDITDFVIRPFVFQANRHFDFNQETAGWSTPRFRPITVTISEKDGAKLGIGVATDFIVPGIPDGWPDTTIGERLVPVGDYAITNSAGIDITTASQYDTAGVIKNNTNFRGMYICGSLQRAWGDKKISNTAFITTATVNRNDLIPSNVIDQTKIAIFQDNHVGVDVQTSDDTLALLGYTGIGEEAIGADRERVVRISTLPETGARGGNHPIFYKNSIKLGYVVRSIDVFNSQILHTSRQLSLNNYLLPPDSFAVYRIIDSNGSWFDIGIDTDGFSFVGVSNIGKLEFPLTASYMGIQLAKIRLASNIRSTMIKL

SEQ ID NO: 40 - protein, 668 aa, Feline calicivirus
MCSTCANVLKYYDWDPHIRLVIDPNRFLSVSFCDKPLLCCYPDLLPEFGTVWDCNQSPLEIYLESILGDDEWSSTFEAIDPVVPPMHWDEAGKIFQPHPGVLMHHLINQVAKAWDPNLPLFRLEADDGSITSPEQGTMVGGVIAEPSAQMSTAADMATGKSVDSEWEAFFSFHTSVNWSTSETQGKILFKQSLGPLLNPYLEHLAKLYVAWSGSVDVRFSISGSGVFGGKLAAIVVPPGVNPVQSTSMLQYPHVLFDARQVEPVIFSIPDLRSTLYHLMSDTDTTSLVIMVYNDLINPYASDSNSSGCIVTVETKPGPDFKFHLLKPPGSMLTHGSVPSDLIPKSSSLWIGNRHWTDITDFVIRPFVFQANRHFDFNQETAGWSTPRFRPITITISEKDGSKLGIGVAMDSIVPGIPDGWPDTTIPEKLVPAGNYAIANGTGNDITTAKDYDSATVIQNNTNFKGMYICGSLQRAWGDKKISNTAFITTATRSDNTITPSNVIDPTKIAVYQDTHVGAEVQTSDDTLAILGYTGIGEEAIGADRDRVVRISVLPETGARGGNHPIFYKNSIKLGYVIRSIDVFNSQILHTSRQLSLNNYLLPPDSFAVYRITDSNGSWFDIGIDSDGFSFVGASNVGKLEFPLTASYMGIQLAKIRLASNIRSSMTKL

SEQ ID NO: 41 - protein, 668 aa, Feline calicivirus
MCSTCANVLKYYGWDPHFRLVVNPNKFLSVGFCDNPLMCCYPDLLPEFGTLWDCDQSPLQIYLESILGDDEWASTYEAIDPSVPPMHWDAMGKIFQPHPGVLMHHIIGEVAKAWDPNLPLFRLEADDGSITAPEQGTVVGGVIAEPSAQMSTAADMATGKSVDSEWEAFFSFHTSVNWSTTETQGKILFKQSLGPLLNPYLEHLAKLYVAWSGSIDVRFSISGSGVYGGKLAAIVVPPGVDPVQSTSMLQYPHVLFDARQVEPVIFSIPDLRSTLYHLISDTDTTSLVIMVYNDLINPYASDTNSSGCIVTVETKPGPDFKFHLLKPPGSMLTHGSIPADLIPKSSSLWIGNRYWSDITEFVVRPFVFQANRHFDFNQETAGWSTPRFRPITVTVSESGGSKLGIGVATDYIVPGIPDGWPDTTIPEKLTPAGNYAITTSNNSDIATATEYDHADEIKNNTNFKSMYICGSLQRAWGDKKISNTAFITTAVKEGNSITPSNTIDMTKLVVYQDAHVGNDVQTSDVTLALLGYTGIGEQAIGSDRDRVVRISVLPETGARGGNHPIFYKNTIKLGYVIRSIDVFNSQILHTSRQLSLNHYLLPPDSFAVYRIIDSNGSWFDIGIDSDGFSFVGVSSLPTLEFPLSASYMGIQLAKIRLASNIRSSMTKL

SEQ ID NO: 42 - protein, 668 aa, Feline calicivirus
MCSTCANVLKYYDWDPHFRLIINPNKFLSVGFCDNPLMCCYPELLPEFGTVWDCDQSPLEIFLESILGDDEWASTYEAIDPVVPPMHWDSAGKIFQPHPGVLMHHLIGEVAKAWDPNLPLFRLEADDGSITTPEQGTSVGGVIAEPSAQMSTAADMATGKTVDSEWEAFFSFHTSVNWSTSETQGKILFKQSLGPLLNPYLTHLAKLYVAWSGSVEVRFSISGSGVFGGKLAAIVVPPGVDPVQSTSMLQYPHVLFDARQVEPVIFTIPDLRSTLYHLMSDTDTTSLVIMVYNDLINPYANDTNSSGCIVTVETKPGPDFKFHLLKPPGSMLTHGSVPSDLIPKSSSLWIGNRYWSDITDFVIRPFVFQANRHFDFNQETAGWSTPRFRPITITISVKESAKLGTGVATDYIVPGIPDGWPDTTIPEELTPAGDYAITNSSGNDITTAAGFDAADVIKNNTNFRGMYICGSLQRAWGDKKISNTAFITTGTVEGGKIRPSNVIDQTKIAVFQDTHANREVQTSDDTLALLGYTGIGEEAIGADRDRVVRISVLPETGARGGNHPIFYKNSIKLGYVIRSIDVFNSQILHTSRQLSLNHYLLSPDSLAVYRITDSNGSWFDIGIDSDGFSFVGVSNIGKLEFPLTASYMGIQLAKVRLASNIRSSMTKL

SEQ ID NO: 43 - protein, 668 aa, Feline calicivirus
MCSTCANVLKYYDWDPHFKLVINPNKFLPIGFCDNPLLCCYPELLPEFGTVWDCGQSPLQIYLESILGDDEWSSTYEAIDPVVPPMHWDEAGKIFQPHPGVLMNYIIGEVAKAWDPNLPLFRLEADDGSITAPEQGTVVGGVIAEPSSQMSTAADMASGKSVDSEWEAFFSFHTSVNWSTSETQGKILFKQSLGPLLNPYLEHLSKLYVAWSGSVEVRFSISGSGVFGGKLAAIVVPPGVDPIQSTSMLQYPHVLFDARQVEPVIFTIPDLRSNLYHLMSDTDTTSLVIMVYNDLINPYANDSNSSGCIVTVETKPGPDFKFHLLKPPGSMLTHGSVPSDLIPRTSSLWVGNRFWGDITDFVIRPFVFQANRHFDFNQETAGWSTPQFRPITVTISVKNGEKLGIGIATDFIVPGIPDGWPDTTIGEELVPAGDYAITTSSGNDITTAQQYDAADIINNNTNFKSMYICGSLQRAWGDKKISNTAFITTATVSGNKLIPSNVIDQTKIAIFQDTHANQGVQTSDDTLAILGYTGIGEEAIGANRERVVRISTLPEAGARGGNHPIFYKNTMKLGYVIRSIDVFNSQILHTSRQLSLNNYLLPPDSFAVYRITDSNGSWFDIGIDTDGFSFVGVSSIGNLEFPLSASYMGIQLAKIRLASNIRSTMTKL

SEQ ID NO: 44 - protein, 668 aa, Feline calicivirus
MCSTCANVLKYYDWDPHIQLVINPNKFLPVGFCDNPLMCCFPELLPEFGTVWDCDQSPLQIYLESILGDDEWASTFEAVEPSVPPMHWDEAGKIFQPHPGVLMHHLIGEVAKAWDPNLPLFRLEADDGSITTPEQGTMVGGVIAEPSAQMSTAADMATGKSVDSEWEAFFSFHTSVNWSTSETQGKILFKQSLGPLLNPYLTHLAKLYVAWSGSIEVRFSISGSGVFGGKLAAIVVPPGIDPVQSTSMLQYPHVLFDARQVDPVIFTIPDLRSTLYHLMSDTDTTSLVIMVYNDLINPYASDSNSSGCIVTVETKPGPDFKFHLLKPPGSMLTHGSVPSDLIPKSSSLWIGNRHWTDITDFVIRPFVFQANRHFDFNQETAGWSTPRFRPITITISVNNAAKLGTGVATDYIVPGIPDGWPDTTIPSELTPAGDYAITNSSGNDITTAVGYDTADEIKNNTNFRGMYICGSLQRAWGDKKISNTAFITTGIVTGNKLQPSNTIDQTKIAVFQDTHANKDPQTSDDTLALLGYTGIGEEAIGADRDRVVRISVLPEAGARGGNHPIFYKNSIKLGYVIRSIDVFNSQILHTSRQLSLNHYLLSPDSFAVYRIIDSNGSWFDIGIDSEGFSFVGVSSIGKLEFPLTASYMGIQLAKIRLASNIRSTLTKL

SEQ ID NO: 45 - protein, 667 aa, Feline calicivirus
MCSTCANVLKYYDWDPHFRLIINPNKFLSVGFCDNPLMCCYPELLPEFGTVWDCDQSPLEIYLESILGDDEWASTYEAIDPVVPPMHWDSAGKIFQPHPGVLMHHLIGEVAKAWDPNLPLFRLEADDGSITTPEQGTSVGGVIAEPSAQMSTAADMATGKTVDSEWEAFFSFHTSVNWSTSETQGKILFKQSLGPLLNPYLTHLAKLYVAWSGSVEVRFSISGSGVFGGKLAAIVVPGVDPVQSTSMLQYPHVLFDARQVEPVIFTIPDLRSTLYHLMSDTDTTSLVIMVYNDLINPYANDTNSSGCIVTVETKPGPDFKFHLLKPPGSMLTHGSVPSDLIPKSSSLWIGNRYWSDITDFVIRPFVFQANRHFDFNQETAGWSTPRFRPITITISVKELAKLGTGVATDYIVPGIPDGWPDTTIPEELTPAGDYAITNSSGNDITTAADFDAADMIKNNTNFRGMYICGSLQRAWGDKKISNTAFITTGTVEGGKIRPSNVIDQTKIAVFQDTHVNQEVQTSDDTLALLGYTGIGEEAIGADRDRVVRISVLPETGARGGNHPIFYKNSIKLGYVIRSIDVFNSQILHTSRQLSLNHYLLSPDSLAVYRITDSNGSWFDIGIDSDGFSFVGVSNIGKLEFPLTASYMGIQLAKVRLASNIRSSMTKL

SEQ ID NO: 46 - protein, 668 aa, Feline calicivirus
MCSTCANVLKYYDWDPHFKLVINPNKFLAVGFCDNPLMCCYPELLPEFGTVWDCNQSPLQIYLESILGDDEWSSTYEAIDPVVPPMHWDEAGKIFQPHPGVLMHHLIGEVAKAWDPNLPLFRLEADDGSITTPEQGTSVGGVIAEPSAQMAAAADMATGKSVDSEWEAFFSFHTSVNWSTTETQGKILFKQSLGPLLNPYLEHLASLYVAWSGSIEVRFSISGSGVFGGKLAAIVVPPGINPVQSTSMLQYPHVLFDARQVEPVIFSIPDLRNSLYHLMSDTDTTSLVIMVYNDLINPYANDTNSSGCIVTVETKPGPDFKFHLLKPPGSMLTHGSIPSDLIPKSSSLWIGNRYWSDITDFIIRPFVFQANRHFDFNQETAGWSTPRFRPITVTISQKEGEKLGIGVATDYIVPGIPDGWPDTTIPGKLTPVGNYAITDESGSDIVTAAEFDSATGIKNNTEFRGMYICGSLQRAWGDKKISNTAFITTAKVNNNMLEPSNVIDQTKIAIFQDNHVGRDVQTSDDTLALLGYTGIGEQAIGSDRDRVVRISILPEAGARGGNHPIFYKNSIKLGYVLRSIDVFNSQILHTSRQLSLNHYLLSPDSFAVYRIIDSNGSWFDIGIDSDGFSFVGVSAIGKLEYPLTASYMGIQLAKVRLASNIRSSMTKL

SEQ ID NO: 47 - protein, 669 aa, Feline calicivirus
MCSTCANVLKYYDWDPHFRLVIDPNKFLSVGFCNNPLMCCYPELLPEFGTVWDCDQAPLQIYLESILGDDEWSSTFEAIDPVVPPMHWNGAGKIFQPHPGILTHHLLSEVAKGWDPNLPLFRLEGDSDSSVTTPEQGTMVGGVIAEPSAQMSTAADMASGKSVDSEWEAFFSFHTSVNWSTSETQGKILFKQSLGPLLNPYLEHLAKLYVAWSGSIEVRFSISGSGVFGGKLAAIVVPPGVNPVQSTSMLQYPHVLFDARQVEPVIFSIPDLRSTLYHLMSDTDTTSLVIMVYNDLINPYANDTNSSGCIVTVETKPGPDFRFHLLKPPGSMLTHGSVPSDLIPKSSSLWIGNRHWTDITDFVIRPFVFQANRHFDFNQETAGWSTPRFRPLTVTISQKDGDKLGTGVATDYIVPGIPDGWPDTTIPGELIPAGDYAITTGNGTDITTAQVFDSADVIQNNTNFRGMYICGSLQRAWGDKKISNTAFITTAIVKGGKLRPSNVIDQTKIAIFQDNHVQAGIQTSDDTLAVLGYTGIGEQAIGADRDRVVRISVLPETGARGGNHPIFYKNSIKLGYVIRSIDVFNSQILHTSRQLSLNHYLLPPDSFAVYRIIDSNGSWFDIGIDSDGFSFVGVSNIGKLEFPLSASYMGIQLAKIRLASNIRSSMTKL

SEQ ID NO: 48 - protein, 668 aa, Feline calicivirus
MCSTCANVLKYYDWDPHFRLIINPNKFLPIGFCDNPLMCCYPDLLPEFGTVWDCDQSPLQIYLESILGDDEWASTHEAIDPSVPPMHWDSAGKIFQPHPGVLMHHLIGEVAKAWDPNLPLFRLEADDGSITTPEQGTAVGGVIAEPSAQMSTAADMASGKSVDSEWEAFFSFHTSVNWSTSETQGKILFKQSLGPLLNPYLEHLSKLYVAWSGSIEVRFSISGSGVFGGKLAAIVVPPGVDPVQSTSMLQYPHVLFDARQVEPVIFTIPDLRSTLYHVMSDTDTTSLVIMVYNDLINPYANDSNSSGCIVTVETKPGPDFKFHLLKPPGSVLTHGSIPSDLIPKSSSLWIGNRYWTDITDFVIRPFVFQANRHFDFNQETAGWSTPRFRPITITISEKNGSKLGIGVATDYIIPGIPDGWPDTTIADKLIPAGDYSITTGEGNDIKTAQAYDTAAVVKNTTNFRGMYICGSLQRAWGDKKISNTAFITTAIRDGNEIKPSNTIDMTKLAVYQDTHVGQEVQTSDDTLALLGYTGIGEEAIGSNRDRVVRISVLPEAGARGGNHPIFYKNSIKLGYVIRSIDVFNSQILHTSRQLSLNHYLLPPDSFAVYRIIDSNGSWFDIGIDSEGFSFVGVSDIGKLEFPLSASYMGIQLAKIRLASNIRSRMTKL

SEQ ID NO: 49 - protein, 668 aa, Feline calicivirus
MCSTCANVLKYYNWDPHIKLSINPNKFLSVGFCDNPLMCCYPELLPEFGTMWDCDQSPLQIYLESILGDDEWASTYEAIDPVVPPMHWDEMGKIFQPHPGVLMHHIIGEVAKGWDPNLPLFRLEADDGSITTPEQGTMVGGVIAEPSAQMSTAADMATGKSVDSEWEAFFSFHTSVNWSTSETQPKILFKQSLGPLLNPYLQHLAKLYVAWSGSIEVRFSISGSGVFGGKLAAIVVPPGVDPVQSTSMLQYPHVLFDARQVDPVIFTIPDLRSTLYHLMSDTDTTPLVIMVYNDLINPYANDSNSSGCIVTVETKPGPDFKFHLLKPPGSMLTHGSVPSDLIPKSSSLWIGNRHWTDITDFVIRPFVFQANRHFDFNQETAGWSTPRYRPITVSISQQEGAKLGIGVAIDYIVPGIPDGWPRSTIPSKLVPAGGYAITAKNGNDITTAAQYDAAGEIVNNTNFKSMYICGALQRAWGDKKVSNTAFVTTATVTGNTLKPSNTIDNTKIAIYQDNHVNSDVQTSDVTLSLLGYTGIGEEAVGADRDKLVRISVLPETGARGGNHPIFYKNSIKLGYVIRSIDVFNSQILHTSRQLSLNNYLLPPDSFAVYRIIDANGSWFDIGIDSDGFSFVGVSNIGKLEFPLSASYMGIQLAKIRLASNIRSTMTKL

SEQ ID NO: 50 - protein, 668 aa, Feline calicivirus
MCSTCANVLKYYGWDPHFRLTINPNDFLSVGFCDNPLMCCYPELLPEFGTVWDCNDSPLQIYLESILGDDEWSSTYEAIDPVVPPMHWDQAGKIFQPHPGVLMHHLLGKVAKGWDPNLPSFRLESDDGSITTPEQGTLVGGVIAEPSTQMATAADMATGKTVDSEWEAFFSFHTSVNWSTSETQGKILFKQNLGPLLNPYLEHIAQLYVAWSGSVDVRFSISGSGVFGGKLAAIVVPPGVQPVQSTSMLQYPHVLFDARQVEPVIFSIPDLRSNLYHLMSDTDTTSLVIMVYNDLINPYANDSNSSGCIITVETKPGPDFKFHLLKPPGSMLVHGSIPSNLIPKSSSLWIGNRHWSDITDFVIRPSVFQANRHFDFKQETAGWSTPRFRPMTITISQKQSAKLGIAVALESIVPGIPDGWPDTTIDSNLIPAGDYAITNQADNDITTAMEYDAATEIKNNTNFRSMYICGALQRAWGDKKVSNTAFITTADLDGNTIKPNNVINQSRIIVYQDNHVNLQVQTSEVTLAMLGYTGIGEEVIGANRDRVVRINVLPEVSARGGNHPIYYKNSLKLGYVIRSIDVFNSQILHTSRQLALNNYLLDPDCFAVYRITDSNGSWFDIGIDYSGFSFVGVSNIGALEFPLTASYTGIQLAKIRLASNIRSSMTKL

SEQ ID NO: 51 - protein, 668 aa, Feline calicivirus
MCSTCANVLKYYGWDPHFDLVINPNDFLSVGFCDNPLMCCYPELLPEFGTVWDCNDSPLQIYLESILGDDEWSSTYEAIDPVVPPMHWKQAGKIFQPHPGHLMHHLIGKVSKGWDPNLPNFRLEADDGSITAPEQGTLVGGVIAEPSAQMSTAADMATGKTVDSEWEAFFSFHTSVNWSTSETQGKILFKQSLGPLLNPYLGHLAQLYVAWSGSVDVRFSISGSGVFGGKLAAIVVPPGVRPVQSTSMLQYPHVLFDARQVEPVIFSIPDLRSSLYHLMSDTDTTSLVIMVYNDLINPYAGDSNSSGCIITVETKPGADFKFHLLKPPGSVLTHGSVPSDLIPKTSSLWIGNRHWADITDFVIRPSVFQANRHFDFKQETAGWSTPRFRPMTVTISQSGGAKLGIGIAHETIVPGIPDGWPDTTIPGELVPAGEYAIVNQTSNDIATAVDYDTATAITNNTNFKSMYICGALQRAWGDKKISNTAFITTADLNGNKIKPNNVINQQRIVIFQDNHVGSEAQTSDVTLAMLGYTGIGEEVIGADRDRVVRINVLPEVSARGGNHPIFYKNTLKLGYVIRSIDVFNSQILHTSRQLALNNYLLDPDSFAVYRITDSNGSWFDIGIDYSGFSFVGVSNIGELEFPLTASYMGVQLAKIRLASNIRSSMTKL

SEQ ID NO: 52 - protein, 668 aa, Feline calicivirus
MCSTCANVLKYYNWDPHFKMVVNPNKFLSVGFCDKPLLCCYPDLLPEFGTVWDCNQSPLEIYLESILGDDEWSSTFEAIDPVVPPMHWDDAGKIFQPHPGVLMHHLISEVAKGWDPNLPLFRLEADDGSITAPEQGTVVGGVIAEPSPQMAVAADTATGKSVDSEWEAFFSFHTSVNWSTSETQGKILFKQSLGPLLNPYLEHLSKLYVAWSGSVEVRFSISGSGVFGGKLAAIVVPPGVDPVQSTSMLQYPHVLFDARQVEPVIFTLPDLRNSLYHLMSDTDTTSLVIMVYNDLINPYANDSNSSGCVVTVETKPGADFKFHLLKPPGSMLTHGSVPSDLIPRSSSLWIGNRYWTDITDFVIRPFVFQANRHFDFNQETAGWSTPRFRPITITISEKNGEKLGIGVATDYIVPGIPDGWPDTTIAEKLTPAGDYAITTGDGNDIITANAYDTADVVKNNTNFRGMYICGSLQRAWGDKKISNTAFITTGTVSDNKIKPSNVIDPTKLAVFQDNHVGADAQTSDDTLALLGYTGIGEHAIGADRERVVRISTLPETGARGGNHPIFYKNSIKLGYVIRSIDVFNSQILHTSRQLSLNHYLLPPDSFAVYRIIDSNGSWFDIGIDSDGFSFVGVTNIGKLEFPLSASYMGIQLAKIRLASNIRSSMIKL

SEQ ID NO: 53 - protein, 668 aa, Feline calicivirus
MCSTCANVLKYYNWDPHFKLVINPNKFLSIGFCDNPLMCCYPELLPEFGTVWDCDQSPLQIYLESILGDDEWSSTYEAIDPVVPPMHWNEAGKIFQPHPGVLMHHIIGEVAKAWDPNLPLFRLEADDGSITAPEQGTVVGGVIAEPSSQMSTAADMASGKSVDSEWEAFFSFHTSVNWSTSETQGKILFKQSLGPLLNPYLEHLSKLYVAWSGSVEVRFSISGSGVFGGKLAAIVVPPGVDPIQSTSMLQYPHVLFDARQVEPVIFTIPDLRSTLYHLMSDTDTTSLVIMVYNDLINPYANDSNSSGCIVTVETKPGSDFKFHLLKPPGSMLTHGSVPSDLIPKTSSLWIGNRFWSDITDFVIRPFVFQANRHFDFNQETAGWSTPRFRPITVTISEKNGAKLGVGVATDFIVPGIPDGWPDTTIGEKLVPAGDYAITNGSGNDITTANQYDAADIIRNNTNFKGMYICGSLQRAWGDKKISNTAFITTATVEGNDLIPSNVIDQTKIAIFQDNHVQDEVQTSDDTLALLGYTGIGEEAIGANRERVVRISTLPETGARGGNHPIFYKNSIKLGYVIRSIDVFNSQILHTSRQLSLNHYLLPPDSFAVYRIIDSNGSWFDVGIDFDGFSFVGVSDVGKLEFPLTASYMGIQLAKIRLASNIRSTMTKL

SEQ ID NO: 54 - protein, 668 aa, Feline calicivirus
MCSTCANVLKYYDWDPHIRLVIDPNRFLSVSFCDKPLLCCYPDLLPEFGTVWDCNQSPLEIYLESILGDDEWSSTFEAIDPVVPPMHWDEAGKIFQPHPGVLMHHLINQVAKAWDPNLPLFRLEADDGSITSPEQGTMVGGVIAEPSAQMSTAADMATGKSVDSEWEAFFSFHTSVNWSTSETQGKILFKQSLGPLLNPYLEHLAKLYVAWSGSVDVRFSISGSGVFGGKLAAIVVPPGVNPVQSTSMLQYPHVLFDARQVEPVIFSIPDLRSTLYHLMSDTDTTSLVIMVYNDLINPYASDSNSSGCIVTVETKPGPDFKFHLLKPPGSMLTHGSVPSDLIPKSSSLWIGNRHWTDITDFVIRPFVFQANRHFDFNQETAGWSTPRFRPITITISEKDGSKLGIGVAMDSIVPGIPDGWPDTTIPEKLVPAGDYAIANGTGNDITTAKDYDSATVIQNNTNFKGMYICGSLQRAWGDKKISNTAFITTATRSDNTITPSNVIDPTKIAVYQDTHVGAEVQTSDDTLAILGYTGIGEEAIGADRDRVVRISVLPETGARGGNHPIFYKNSIKLGYVIRSIDVFNSQILHTSRQLSLNNYLLPPDSFAVYRITDSNGSWFDIGIDSDGFSFVGASNVGKLEFPLTASYMGIQLAKIRLASNIRSSMTKL

SEQ ID NO: 55 - protein, 668 aa, Feline calicivirus
MCSTCANVLKYYDWDPHFRLNVNPNEFLSVGFCDKPLMCCYPELLPEFGTVWDCSRAPLEIYLESILGDDEWSSTHEAIDPVVPPMHWDEAGKIFQPHPGVLMHHLINKVARAWDPNLPLFRLEADDGSITTPEQGTLVGGVIAEPSSQMSAAADMATGKSVDSEWEAFFSFHTSVNWSTSETQGKILFKQSLGPLLNPYLEHLSKLYVAWSGSVEVRFSISGSGVFGGKLAAIVVPPGVDPVQSTSMLQYPHVLFDARQVDPVIFTIPDLRSNLYHLMSDTDTTSLVIMVYNDLINPYANDSNSSGCIVTVETKPGPDFKFHLLKPPGSMLTHGSVPSDLIPKSSSLWIGNRHWTDITDFVIRPFVFQANRHFDFNQETAGWSTPRFRPLSVTISQSGGAKLGIGIATDYIVPGIPDGWPDTTIPGELTPAGDYAIVNQNNSDIATKQAYESATSIENNTNFKSMYICGSLHRAWGDKKISNTAFITTATVDGNNLIPSNTIGQDKIAVFQDNHVNAEVQTSDVTLATLGYTGIGEEAIGAIRDRVVRISVLPETGARGGNHPIFYKNAMKLGYVIGDIDVFNSQILHTSRQLSLNNYLLPPDSFAVYRIIDSNGSWFDVGIDSDGFSFVGVSSIPKLEFPLSASYMGIQLAKIRLASNIRSTMTKL

SEQ ID NO: 56 - protein, 671 aa, Feline calicivirus
MCSTCANVLKYYGWDPHFKLVINPNNFLPVGFCSNPLMCCYPELLPEFGTVWDCDRSPLEIYLESILGDDEWASTFDAVDPVVPPMHWSAAGKIFQPHPGVLMHHLIGKVAAGWDPDLPLIRLEADDGSITAPEQGTMVGGVIAEPSAQMSTAADMATGKSVDSEWEAFFSFHTSVNWSTSETQGKILFKQSLGPLLNPYLEHLAKLYVAWSGSIEVRFSISGSGVFGGKLAAIVVPPGVDPVQSTSMLQYPHVLFDARQVEPVIFSIPDLRSTLYHLMSDTDTTSLVIMVYNDLINPYANDANSSGCIVTVETKPGPDFKFHLLKPPGSMLTHGSVPSDLIPKTSSLWIGNRYWSDITDFVIRPFVFQANRHFDFNQETAGWSTPRFRPISVTISQQDGAKLGIGVATDYIVPGIPDGWPDTTIPGELIPAGDYAITNNIGDDITTATGYDTADIIKNNTNFKGMYICGSLQRAWGDKKISNTAFITTATLSGNNNNKINPCNTIDQSKIVVFQDNHVGKEVQTSDDTLALLGYTGIGEQAIGSDRDRVVRISTLPETGARGGNHPIFYKNSIKLGYVIRSIDVFNSQILHTSRQLSLNHYLLPPDSFAVYRIIDSNGSWFDIGIDSDGFSFVGVSGFGKLEFPLSASYMGIQLAKIRLASNIRSPMTKL

SEQ ID NO: 57 - protein, 668 aa, Feline calicivirus
MCSTCANVLKYYDWDPHIRLVINPNKFLPIGFCDNPLMCCYPELLPEFGTVWDCDQSPLQIYLESILGDDEWASTYDAIDPVVPPMHWDDAGKIFQPHPGVLMHFLINEVAKGWDPSLPSFRLEADDGSITTPEQGTAVGGVIAQPSAQMSAAADMASGKSVDSEWEEFFSFHTSVNWSTTETQGKILFKQSLGPLLNPYLEHLSKLYVAWSGSIDVRFSISGSGVFGGKLAAIVVPPGVDPVQSTSMLQYPHVLFDARQVEPVIFSLPDLRNSLYHLISDTDTTSLVIMVYNDLINPYANEANSSGCIVTVETKPGPDFKFHLLKPPGSMLTHGSIPSDLIPRSSSLWIGNRHWTDITDFVIRPFVFQANRHFDFNQETAGWSTPRFRPITINISQKEGARLGTAIAVDTILPGIPDGWPDTTIPTVLTPAGKYAITSGNNSDILTRNDYENADVIKNNTNFRSMYICGSLQRAWGDKDISNTAFITTGTVNGNNIEPSNTIDPTKLAVFQDNHVKSEVQTSDVTLSVLGYTGIGEEAVGADRDKVVRISVLPETGARGGNHPIFYKNSMKLGYVISSIDVFNSQILHTSRQLSLNHYLLPPDSFAVYRITDSNGSWFDIGIDNDGFSFVGVSHIGKLEFPLSASYMGIQLAKIRLASNIRSSMIKL

SEQ ID NO: 58 - protein, 668 aa, Feline calicivirus
MCSTCANVLKYYDWDPHFRLVIDPNKFLSVGFCDNPLMCCYPELLPEFGTVWDCDQSPLQIYLESILGDDEWASTYEAIDPSVPPMHWDSAGKIFQPHPGVLMHYIIGEVAKAWDPNLPNFRLEADDGSITTPEQGTMVGGVIAEPSAQMATAADTATGKSVDSEWEAFFSFHTSVNWSTSETQGKILFKQSLGPLLNPYLTHLAKLYVAWSGSIEVRFSISGSGVFGGKLAAIVVPPGIDPVQSTSMLQYPHVLFDARQVEPVIFTIPDLRSTLYHLMSDTDTTSLVIMVYNDLINPYANDSNSSGCILTVETKPGPDFKFHLLKPPGSMLTHGSVPSDLIPKSSSLWIGNRYWSDINDFVIRPFVFQANRHFDFNQETAGWSTPRFRPITVTISVKESAKLGIGVATDYIVPGIPDGWPDTTIPTDLTPAGDYAITDSTGNDITTPSGYDSAISIVNNTNFRGMYICGSLQRAWGDKKVSNTAFITTGIVTGNKLEPSNTIDQTKIAIFQDTHANRDTQISDDTLALLGYTGIGEEAIGADRDRVVRISVLPETGARGGNHPIFYKNSIKLGYVIRSIDVFNSQILHTSRQLSLNHYLLSPDSFAVYRITDSNGSWFDIGIDSDGFSFVGVNNIGKLEFPLTASYMGIQLAKIRLASNIRSTMTKL

SEQ ID NO: 59 - DNA, 7685 bp, Feline calicivirus
gtaaaagaaatttgagacaatgtctcaaactctgagcttcgtgcttaaaactcacagcgtccgcaaggactttgtgcactccgtcaagctaacgcttgcacggaggcgcgatcttcagtatttctataacaagctctctcgttctatgcgagctgaagcttgtccttcttgtgccagttatgatgtatgtcctaactgcacttctagtgatatccctgatgatggttcatcaacaacgttgatgccatcatgggaggatgtcacaaaaacctctacttactctcttctactctccgaagatacttctgacgagttgtctcctgacgaattggttcacgttgctgctcacattcgcaaggcgctttccactcagtctcatccggccaatgttgacatgtgcaaagaacagctcacgtcattattggtgatggctgaagctatgctgcctcaacggtcacgagcaacaatcccacttcatcaacaacaccagacggctcgcattgaatggagggaaaagttcttctctaagccccttaacttcattcttgaaaagattggtgtttctaaagatattcttcaggttactgccctttggaaaatcatcttggagaaagcttgctactgcaaatcctatggtgaagagtggttcgatgctgcaaagaacaaactaagggagatgagaagcttcgaaagcaacacactcaaaccactggttggagctttcattgacggcttaaggtttatgactgtggataaccccaaccctatggcattcttacccaagctaattgggcttatcaaacccctcaatttggcaatgataatcgacaatcatgaaaacacactatcaggatggatcattaccctcactgcaattatggagttatacaacatcacagaatgcacaattgacataatcacttcactggtaacagcattctatgacaaaattgctaaagcccctaaattctacagtcagatcaaagcactgttcacgggatttaggacagaggatgtggctaattcattttggtatatggctgctgcaattctatgttacctgattacgggtataatcccaaacaatgggaggttttcaaagattaaaacctgcctgtctggtgcaacgaccctggtatcgggtataattgccacacagaaacttgcagcaatgttcgctacatggaactctgaatccattgttaacgaattatctgcaaggacagtggctatttctgaattgaataacccaactactacctctgacactgactctgttgagcggttgctcgaattggctaagatcttgcacgaggagatcaaagttcacactctgaatccaattatgcaatcatacaacccaattcttagaaatttaatgtccacactagacggtgttgtcacctcatgcaacaagagaagagcaattgccaaaaagaggcaagtcccagtttgctacatccttactggaccacctggatgtggcaagaccactgcggccctagcccttgcaaagaagctctctgatcaagagccatcagtgattaatttggatgttgatcatcatgatacttacactggcaatgaagtgtgcattgttgatgagtttgattcatcagacaaagtggactatgcaaattttgtgattggtatggttaattcggcaccaatggttctaaattgtgatatgcttgaaaataagggaaagctctttacctctaagtacataataatgacttctaactctgaaacccctgtaaaaccctcttctaagcgtgcaggtgctttctaccgaagagttacaatcattgacgttgcaaaccctttggtggaatctcacaagcgcgcgcgccctggaacatctgtccctcgaagctgctacaagaagaacttttcacacctttcacttgctaaacgaggggctgagtgctggtgcaaggagtatgttttggaccccaagggacttcagcatcagagtatcaaggctcctcctcccacttttcttaacattgattcccttgcccaaactatgaaacaagacttcattcttaagaacatggcatttgaggcagagaatggctctagtgagcacaggtttggctttgtctgtcagcagagtgaggtcgacactgttcgcaggctgcttaatgcaataagggcacggcttaacgcgacattcactgtgtgcgttgggcctgagtcctcaaattccattgggtgtactgctcatgtcctcactcccgatgagcctttcaatgggaagaggtttgttgtatctcgatgcaacgaagcctcccttgcagcactagaaggaaattgcgtgcagactgcgttgggcgtatgcatgtccaacaaggatttaacccacctgtgccatttcataagagggaagattgtcaatgatagtgtcaggctggacgaactacccgccaatcaacatgtggtaaccgtgaattcggtatttgatttggcctgggctcttcgccgtcacctcacactatctggacagtttcaagcaatcagagccgcatatgatgtgctaactgtccccgacaaaattccagctatgttaaggcactggatggatgaaacatccttttcggatgagcatgtagtcacacagtttgtaacgccaggtggtattgtcatcttggaatcatgtggtggagcacgtatctgggctttgggtcacaatgtgatccgcgctggaggtatcactgcaacaccaactggtggttgtgtcagattaatgggtctctctgccccttctatgccatggtctgaactctttcgagaacttttctctttattgggtaggatatggtctagtgttaaagtctccactcttgttctgaccgctcttggaatgtacgcatctagatttagacccaaatcagaagctaagggaaaaacaaaatccaaggttgggccctacagaggtcgtggtgtagcgctcactgatgatgagtacgatgaatggagggaacacaacgccacacgaaaattggacttatcagtagaagattttctgatgctgcgccatcgtgcagcacttggtgctgatgatgcagatgcagttaaatttagatcatggtggaactcaagatcaaaattggcggatgattttgaagatgtcaccgtgattggaaaaggtggtgttaaacatgaaagaatcagaacaaacaatctcagagctgtggagcgtggatatgacgttagctttgctgaagaatcaggacccggcacaaaattccacaaaaacgccattggatctgtaactgatgtttgtggtgagcacaagggatactgtgtccatatgggtcatggggtgtacgcctcagtagcccatgtggtgaaaggtgattcattctttcttggtgagagaatatttgacctcaaaactaatggtgagttttgctgctttcgcagtacaaagatcttgcccagtgctgcgcctttcttctcaggcaaacccacccgtgacccgtggggctcacctgttgccacagaatggaagccaaaaccatacaccactacatcagggaagattatagggtgttttgctacaacttcaactgaaacccacccaggtgattgtggtctaccttacatcgatgacaatggtagagtcactggactgcacacaggatccggtggacccaaaactcccagcgcaaaattggttgtcccctatgtccatattgatatgaaaacaaaatctgttactgcccaaaagtatgacattacaaagcctgatattagttacaaaggattgatttgcaaacaattggatgaaattcggataataccaaaaggaacacgcctccacgtttctcctgcccacacagatgattatgaggaatgttcgcaccaaccagcatcactaggtagtggtgatccacgatgtccaaaatcccttactgctattgtagttgactccttaaaaccctactgtgataaggttgagggccccccccatgatgttttgcatagggttcagaaaatgctaattgatcacctctctggctttgttcctatgaatatctcttctgaaaactcaatgctctctgcatttcacaaactcaatcatgatacatcctgtggcccatacttaggtggaagaaagaaagatcatatggtaaatggtgagcctgacaaggcactgttggatttgctatcttcaaaatggaaacttgccactcaagggattgctctccctcatgagtacacaattgggctaaaagatgaattgagaccaattgagaaagttcaggaaggaaagagaaggatgatctggggttgtgatgttggggttgccacagtttgcgctgctgcatttaaaggtgttagtgacgcaataacggcaaaccaccagtatggacctgttcaagttgggattaacatggatagccccagtgttgaggcactttaccaacgaatcaagagcgctgccaaggtttttgcggtcgattactccaagtgggattcgactcaatcgcctcgggttagtgctgcctcaattgatattcttagatacttctctgatagatctccaattgttgattcagctgcaaacaccttaaaaagtcctccaatagcggtgttcaatggtgttgcagtaaaggtttcgtctggtcttccatctggtatgcctctgacttctgtaattaactctttaaatcactgcctatatgttggttgtgctatccttcaatctctggaatccaaaaacatacctgtcacttggaatctgttctcctcatttgacatgatgacttacggtgatgatggtgtttacatgttccctatcatgtttgctagtgttagtgatcaaatctttggaaaccttactgcttatggcttaaaacccacaagggtcgacaaatcagttggagctattgaaccaatcgatcctgaatctgttgttttcctaaaaagaaccatccaaaggacccctagtggcattcgaggtcttcttgatcgcagctcaatcctcagacagttctattacattaaaggtgaaaattcggatgattggaaaactcctccaaaagtcatagatcccacctccagaggtcaacagctgtggaacgcttgtctttatgctagccaacatggtgttgagttttacaataaggttctcaaattggcccagaaagctgttgaatacgaaggattacacctcgaccccccaagcttccaatcggcattggaacattacaataaccaatttagtggtgtggaggcgcggaatgaccagatcgattcgagtggcatgtccgccctacactgtgatgtgttcgaagtttgagcatgtgctcaacctgcgctaacgtgcttaaatactatgattgggatccccacttcaaattggtgatcgaccctaataaatttctttctgttggattctgtgataacccgcttatgtgttgctatcctgagttgcttccagaattcggcactgtgtgggattgtgatcaatctccactgcaaatttaccttgaatctattcttggtgatgatgaatggtcttctacctatgaagccattgaccctgtcgttccaccaatgcactgggacaaaatggggaaaatcttccaacctcaccctggtatgctaatgcaccatatcatcggtgaagttgccaagggatgggatccaaacttgcctttgttccgattggaggccgatgatggatcggtgacaacccctgaacaaggaacaatggttggcggagtcattgctgaacccagcgcccaaatgtcaactgctgctgacatggcctctgggaaaagtgttgactccgaatgggaggctttcttctcatttcacactagtgtaaattggagtacatctgaaacacaaggaaagattctattcaaacaatcacttggacccctgctaaacccatatcttgaacacatatctaagctttatgttgcatggtctggatctatagaggttaggttttctatttctggttctggtgtttttgggggaaaactcgctgctattgttgtgccgcctggggtagacccagtgcaaagcacatcaatgctacagtatcctcatgttctatttgatgcccgtcaggtagaacctgttatcttttcaatacctgatttgagaaacagcttgtaccatcttatgtcagatactgatactacctcccttgtaattatggtgtacaatgatcttattaatccttatgcaaatgattctaactcttctggatgtattgtcactgttgagactaaacctggaatcgatttcaagtttcaccttctgaaaccccctggatctatgcttacccatggctctatcccttcagatttaataccaaaatcttcttctctttggatagggaatcgtcactggactgacataaccgattttgtcattaggccttttgtgttccaagcaaaccgtcattttgattttaatcaggaaacagctggttggagtacgccaagattccgaccactagccgtaacggttagccaaagtaaaggagcaaaattggggaatggtattgcgaccgactacatcgtgcctgggattcctgatggatggccagacactacaatcccaacaaaactgacacccacaggcgattatgcaattacatctagtgatggtaatgacattgaaacaaaacttgaatacgaaaatgctgatgtgattaaaaacaacacaaacttcaggagcatgtacatttgtgggtcgctccaaagagcctggggtgataagaagatttctaatactggtttcataactactggtgttatctctgataattccataagcccaagcaataccattgatcaaagcaaaatcgtggtctatcaagacaatcatgtcaatagtgaagttcaaacctcagacatcacacttgcaattcttggctacactggtattggtgaggaggcaattggcgccaatcgggactcggttgtacgcataagtgtgctgccagaaacaggtgcccgtgggggaaaccatccaatcttttataagaattctatgaagcttggttacgtgatcagctccattgatgtgtttaattcccagatcttgcacacctctagacaactatcactgaataactacttactacctccagattcttttgctgtctatcgaattattgattctaatgggtcttggtttgatataggcattgattctgatggattttcttttgttggtgtctcaagttttcctaagttagagtttccactttctgcctcctatatgggaattcagttggcaaagattcgtcttgcctctaatattaggagttctatgactaaattatgaattcaatattaggcttaattgacactgttacaaatacaattggcaaagctcaacaaattgaattagataaagctgcacttggtcaacaacgcgaactggctttgcaacgaattaaccttgatcgccaggcgttgaacaaccaagttgagcaatttaacaaaattcttgagcaaagggtacaaggccccatccagtctgtgcggctcgcacgtgctgctggatttagggttgacccttactcatacacaaatcaaaatttttacgatgaccaattgaatgcaattagactatcttataggaatttgtttaaataattggccacaagtatcccttcgggctgccgcatttgcgcctaaccccagggc

SEQ ID NO: 60 - DNA, 7690 bp, Feline calicivirus
gtaaaagaaatttgagacaatgtctcaaactctgagcttcgtgcttaaaactcacagtgtccgaaaggactttgtgcactctgtcaagttaacacttgcacggaggcgcgatcttcagtatatttataacaagctctcacgcactatacgtgctgaggcttgcccttcttgtgctagttacgacgtatgtcctaactgcacctctggtgacgtcccggatgacgggtcttcgacaatgtcgattccatcatgggaggatgtcacaaagtcttcaacctactctctcctgctctctgaggacacctccgacgagttatgccctgaggacttggttaatgtggctgctcatatccgtaaggcgctatccactcagtcccacccggctaatgctgaaatgtgcaaagaacagctcactttcttattagtcatggctgaggcgatgctgccccaacgatcccgagcgtcaatcccactgcaccaacaacacacggctgcacggttggaatggagggagaaattcttctctaaacctcttgactttctccttgaaagagttggtgtgtcaaaagatattctccaaactactgcgatttggaaaattatcttggaaaaagcatgctattgtaaatcctatggagagcagtggttcactgctgccaaacaaaagttaagggaaatgaaaaactttgagagtgatacgctaaaacctcttattggtggatttatagatggtctacggttcttgaccgtggacaacccaaacccgatgggtttcctcccaaaactcatagggcttgtaaaacccctgaatttggcgatgattattgataatcatgaaaacacaatatctggctggatcatcacattaaccgcaataatggagctatacaacatcaccgaatgcaccatagatattataacatcagtcattacggctttctatgataaaattggcaaggcaaccaaattttacagttgtgttaaggcgctgttcactggatttagatctgaggacgtagcgaattccttttggtacatggcagcagcgattctatgttacctgatcactgggttaatcccaaacaacggcagattttcaaagataaaagcttgcctggccggagcgacaactcttgtatcaggtatagttgccacacaaaagctagctgcaatgttcgcaacatggaactctgagtccattgttaatgagttgtcagcaagaactgttgccctatcagagctaaacaatccaacaacaacgtctgacacggattcggtagaacgactgctagaattggctaagatcttgcatgaggagatcaagattcatactctaaaccccatcatgcaatcatacaatccaatcttgagaaatttaatgtcaaccttggacggtgttataacatcatgcaacaagaggaaagctattgctcggaagagacaggtgccagtttgttacatattaactggcccacctggatgtgggaaaacaaccgcagctcaagcattagctaagaaattgtctgatcaagagccgtcggtaattaaccttgatgttgatcatcatgacacatatactggaaatgaggtatgtatcattgatgagtttgattcgtctgacaaggtagactatgcaaattttgtgattgggatggtaaactctgctcctatggtgttaaattgtgacatgcttgagaacaagggaaagctcttcacctcaaagtatataattatgacttccaactctgaaactccagtgaaaccctcttccaagcgcgcaggtgcattctaccgaagggttactatcatcgatgtaactaacccttttgtggagtcgcacaagcgtgcaaggcctgggacgtctgttcctcgtagctgctataagaaaaacttctcccatctctcacttgctaaacgaggggccgagtgctggtgcaaggaatacgttcttgaccctaaggggcttcaacaccaaagcatgaaggctccccctcctacctttcttaacattgactctttagctcagacgatgaagcaagacttcttgctcaagaacatggcttttgaggctgaagatgggtgcgcagaacatcgatatgggtttgtgtgtcaacaggaagaggttgaaactgttcgcaggctcctcaacgcggttagggcaaggatgaatgctaccttcactgtgtgtgttggacccgagacctcgcactcgattggttgcactgcgcacgtgttaactcccaatgagacctttaatggaaagaagtttgttgtgtcacgatgtaacgaagcatcactttctgcccttgaaggtaactgtgtaaagtcagctttgggcgtgtgtatgtcagataaggatctcactcatttatgccacttcattaaagggaaaattgtcaatgacagtgttaggttggatgaactacccgccaatcagcatgtggtaaccgttaattcggtgtttgatttggcctgggctgttcgtcgtcatctcacactggcagggcagtttcaagctatcagagccgcatatgatgtgcttactgtccccgacaagatccctgcaatgttgcgtcactggatggatgagacctccttttctgatgaccacgttgtaacacaatttgtaacacctggtggcatagtcatcctggagtcttgcggtggtgcacgcatctgggctttaggtcgcaacgtgatccgagcaggaggtgtcaccgcaaccccaaccggaggatgtgttaggttaatgggattatctgcgccaaccatgccatggtccgagatctttcgtgagctcttctctctcttaggtagaatttggtcatctgtcaaagtatcagccctagtactaactgctcttggaatgtacgcatctagatttagaccaaaatcggaagcaaaaggaaaaaccaaattgaagattgggacatacaggggtcgcggtgtagcgctgactgatgacgagtacgatgagtggcgcgaacacaacgcctccagaaaattggatttgtcagtggaggatttcttaatgttgcgccatcgtgccgctctaggagccgacgacaatgatgcagtaaaattccggtcgtggtggaactccagaaccaaaatggccaatgattatgaggatgtcaccgtaattggcaaaggtggcgtcaaacatgaaaagatcagaaccaataccctaaaagctgtggatcgtggttatgacgtcagctttgctgaggaatcaggaccaggcaccaagttccacaagaatgcaattggatctgtcacagatgtttgtggggagcacaaaggctattgcatccacatgggccacggtgtttacgcatccgtagctcacgtggtgaaaggggattcatttttcttgggtgaaaggatttttgatcttaagactaatggtgaattttgctgctttcgcagcacgaaaattctacctagtgctgcacctttcttttctgggaagcccactcgtgatccgtggggatcccccgtggcaactgagtggaagcctaaaatgtacacaacaacctctggaaagattctggggtgctttgcaacaacttcaactgaaactcacccgggagactgtggcctcccatatattgatgacaacgggagggtgaccggcctccacactggctctgggggacccaaaaccccaagtgccaagttggtggtgccatatgtgcatattgacatgaagactaaatccgtcactgctcaaaagtatgacgtaacaaagcctgatataagttacaaaggcttaatttgtaagcaattggatgagattaggattataccaaaaggcacacgtctccatgtctccccagcccacactgaggattatcaagaatgctcacaccaacccgcatcacttggaagcggggatccccgctgtccaaaatctctcactgctatagttgttgattctctaaaaccatactgtgagaacgttgagggtcctccacatgatgttttgcacagagttcaaaagatgcttatcgaccacctttcaggctttgtccctatgaacatttcctcggaaacctctatgctctcagctttccacaaactcaatcatgatacttcctgtggaccatacttgggtggcagaaagaaagatcacatggctaacggtgagccggacaagcagttattggatctcctgtctgcaaaatggaaattggcaacccaaggcatagcactaccacatgagtacacaattgggctaaaggacgagttaaggcccgtggagaaggttagtgaagggaagagaaggatgatttggggttgtgatgttggcgtcgctactgtctgtgcagctgcgttcaagggtgttagcgatgccatcacagcaaaccaccagtacgggcctatacaggttggtatcaacatggatagccccagcgtcgaagcgctgttccaaaggatcaaaagcgcggccaaggtatttgcggtcgattattccaaatgggattcgacccaatcgcctcgtgtcagtgcagcttcaattgacatccttcgttacttttccgatcgctctccaattgttgactcagcctctaacacactgaagagccctcctgttgcaatctttaatggtgttgctgtaaaagtgtcctctggcttaccatctggaatgcctcttacctcagtaatcaattcccttaatcattgtctgtatgttgggtgtgccattcttcaatccctagaagctaaggccattcccgtcacttggaaccttttctcaacttttgatatcatgacttacggggatgatggtgtctacatgtttcctattatgtatgcaagtattagtgaccaaatttttggaaatctttcttcctatggcctgaaaccaactcgggttgacaagtccgttggagcaattgagcctattgatcctgactctgttgttttcttgaagagaacaatcacaaggacacctcaggggataaggggtttacttgatcgcagctctataataagacaattctattatattaaaggtgagaactccgatgactggaagagccccccaaaacatattgacccaacatctcgagggcaacagctttggaatgcctgtctgtacgctagccaacatggcttggagtttttcaacaaggtttacaggctggccgagagggctgttgaatatgaagagctgcactttgaacccccaacatatgcttcggctttggatcattacaacagccagttcaatggcgtggaggcgcggtctgaccagatcgactcgagtggcatgaccgccctacactgtgatgtgttcgaagtttgagcatgtgctcaacctgcgctaacgtgcttaaatattatgattgggacccccatttcaaattggtaatcaaccccaacaacttcctctctgttggcttttgtagtaaccctttaatgtgttgctacccagaactccttccggaatttggaactgtttgggattgcgatcggtcaccacttgaaatttacctagaatcaatacttggtgatgatgaatgggcatccacttttgacgctgttgacccagtcgttcccccaatgcactggggtgctgctggaaaaattttccagccacaccccggtgttctcatgcaccatctcattggtaaggttgctgcaggttgggaccccgatctgcctctaattcgactcgaggcggatgacgggtcaatcacagcacccgagcaaggaacaatggttggcggcgtcatcgctgaacccagcgcccagatgtcaacagctgctgatatggccaccgggaaaagcgttgattctgagtgggaggcattcttctcctttcacaccagcgtcaattggagtacatctgaaacccaaggaaagattctcttcaaacaatccttaggccctttgctcaacccatatctagaacaccttgctaagctatatgttgcgtggtctgggtcgattgaggttaggttctctatctctggctctggtgtctttggtgggaagctcgcagctattgttgtacctcctggggttgatccagtgcagagtacttcgatgctacaatacccccatgttttgtttgatgctcgtcaggtggaaccagttatcttctgtcttcctgatctaagaagcaccctgtaccaccttatgtctgacactgacactacatccttggtcattatggtgtacaatgatctcatcaatccctatgccaatgatgccaactcttctgggtgtattgtcactgtcgagacaaaacctggccctgacttcaagtttcacctccttaagccacccggatctatgctaacccatggctctatcccttctgatttaattcccaaaacatcttcgctctggatcggtaaccgctactggtcagacataactgattttgtgattcggccgtttgtcttccaagcaaatcgtcattttgactttaatcaagagaccgcagggtggagcacaccacggtttcggcctatatctgttaccattactgaacagaacggagcaaaattgggcattggggtggcaacagattacatagtgcctggaatccctgatggctggcctgacaccacaattcctggggagttgataccagctggtgattacgcaatcaccaatggtactggcaatgacatcaccacggctacaggatatgacactgctgatataattaagaacaataccaactttaggggcatgtacatatgtggttcgctccagcgtgcctggggtgataagaaaatttccaacactgcctttatcaccactgccaccctagatggtgacaacaacaacaagatcaatccctgtaataccatagaccagtcaaagatcgtcgtgtttcaagacaaccatgttggaaagaaagcgcaaacctcagacgatacattggccctgcttggttacactggcattggtgagcaggccatcgggtctgatagggaccgggttgtgcgcatcagcactctccctgaaactggtgctcgaggcggtaaccacccaattttctacaagaactccattaaattgggatatgtaattaggtctattgatgtctttaattcacaaatcttgcacacttccagacagttatcgctaaatcattacctactcccacctgattcttttgccgtctatagaataattgactcaaatggctcgtggtttgatattggaattgatagtgatgggttctcttttgttggtgtttctggctttggtaaattagaatttcccctttctgcctcctacatgggaatacaattggcaaagatccggcttgcctctaacattaggagtcccatgactaagttatgaattcaatattaggcctgattgatactgttactaacactattggtaaagctcagcagattgaattggacaaagctgcacttggtcaacagcgtgaattggctctccagcgcattggcttggaccgccaagccttaaacaaccaagttgagcagtttaacaaaattcttgagcaaagggtacaaggcccaatccaatccgttcgccttgcgcgcgcggctggatttagggttgacccttactcatacacaaaccaaaacttttatgacgatcaattaaatgcaattagactatcatataaaaatttgtttaaaatttgatcatatatccctttgggctgccgcacctgcgcctaaccccaggg

SEQ ID NO: 61 - DNA, 7690 bp, Feline calicivirus
gtaaaagaaatttgagacaatgtctcaaactctgagcttcgtgcttaaaactcacagcgtccgcaaggactttgtgcactccgtcaagctaacgcttgcacggaggcgcgatcttcagtatttctataacaagctctctcgttctatgcgagctgaagcttgtccttcttgtgccagttatgatgtatgtcctaactgcacttctagtgatatccctgatgatggttcatcaacaacgttgatgccatcatgggaggatgtcacaaaaacctctacttactctcttctactctccgaagatacttctgacgagttgtctcctgacgaattggttcacgttgctgctcacattcgcaaggcgctttccactcagtctcatccggccaatgttgacatgtgcaaagaacagctcacgtcattattggtgatggctgaagctatgctgcctcaacggtcacgagcaacaatcccacttcatcaacaacaccagacggctcgcattgaatggagggaaaagttcttctctaagccccttaacttcattcttgaaaagattggtgtttctaaagatattcttcaggttactgccctttggaaaatcatcttggagaaagcttgctactgcaaatcctatggtgaagagtggttcgatgctgcaaagaacaaactaagggagatgagaagcttcgaaagcaacacactcaaaccactggttggagctttcattgacggcttaaggtttatgactgtggataaccccaaccctatggcattcttacccaagctaattgggcttatcaaacccctcaatttggcaatgataatcgacaatcatgaaaacacactatcaggatggatcattaccctcactgcaattatggagttatacaacatcacagaatgcacaattgacataatcacttcactggtaacagcattctatgacaaaattgctaaagcccctaaattctacagtcagatcaaagcactgttcacgggatttaggacagaggatgtggctaattcattttggtatatggctgctgcaattctatgttacctgattacgggtataatcccaaacaatgggaggttttcaaagattaaaacctgcctgtctggtgcaacgaccctggtatcgggtataattgccacacagaaacttgcagcaatgttcgctacatggaactctgaatccattgttaacgaattatctgcaaggacagtggctatttctgaattgaataacccaactactacctctgacactgactctgttgagcggttgctcgaattggctaagatcttgcacgaggagatcaaagttcacactctgaatccaattatgcaatcatacaacccaattcttagaaatttaatgtccacactagacggtgttgtcacctcatgcaacaagagaagagcaattgccaaaaagaggcaagtcccagtttgctacatccttactggaccacctggatgtggcaagaccactgcggccctagcccttgcaaagaagctctctgatcaagagccatcagtgattaatttggatgttgatcatcatgatacttacactggcaatgaagtgtgcattgttgatgagtttgattcatcagacaaagtggactatgcaaattttgtgattggtatggttaattcggcaccaatggttctaaattgtgatatgcttgaaaataagggaaagctctttacctctaagtacataataatgacttctaactctgaaacccctgtaaaaccctcttctaagcgtgcaggtgctttctaccgaagagttacaatcattgacgttgcaaaccctttggtggaatctcacaagcgcgcgcgccctggaacatctgtccctcgaagctgctacaagaagaacttttcacacctttcacttgctaaacgaggggctgagtgctggtgcaaggagtatgttttggaccccaagggacttcagcatcagagtatcaaggctcctcctcccacttttcttaacattgattcccttgcccaaactatgaaacaagacttcattcttaagaacatggcatttgaggcagagaatggctctagtgagcacaggtttggctttgtctgtcagcagagtgaggtcgacactgttcgcaggctgcttaatgcaataagggcacggcttaacgcgacattcactgtgtgcgttgggcctgagtcctcaaattccattgggtgtactgctcatgtcctcactcccgatgagcctttcaatgggaagaggtttgttgtatctcgatgcaacgaagcctcccttgcagcactagaaggaaattgcgtgcagactgcgttgggcgtatgcatgtccaacaaggatttaacccacctgtgccatttcataagagggaagattgtcaatgatagtgtcaggctggacgaactacccgccaatcaacatgtggtaaccgtgaattcggtatttgatttggcctgggctcttcgccgtcacctcacactatctggacagtttcaagcaatcagagccgcatatgatgtgctaactgtccccgacaaaattccagctatgttaaggcactggatggatgaaacatccttttcggatgagcatgtagtcacacagtttgtaacgccaggtggtattgtcatcttggaatcatgtggtggagcacgtatctgggctttgggtcacaatgtgatccgcgctggaggtatcactgcaacaccaactggtggttgtgtcagattaatgggtctctctgccccttctatgccatggtctgaactctttcgagaacttttctctttattgggtaggatatggtctagtgttaaagtctccactcttgttctgaccgctcttggaatgtacgcatctagatttagacccaaatcagaagctaagggaaaaacaaaatccaaggttgggccctacagaggtcgtggtgtagcgctcactgatgatgagtacgatgaatggagggaacacaacgccacacgaaaattggacttatcagtagaagattttctgatgctgcgccatcgtgcagcacttggtgctgatgatgcagatgcagttaaatttagatcatggtggaactcaagatcaaaattggcggatgattttgaagatgtcaccgtgattggaaaaggtggtgttaaacatgaaagaatcagaacaaacaatctcagagctgtggagcgtggatatgacgttagctttgctgaagaatcaggacccggcacaaaattccacaaaaacgccattggatctgtaactgatgtttgtggtgagcacaagggatactgtgtccatatgggtcatggggtgtacgcctcagtagcccatgtggtgaaaggtgattcattctttcttggtgagagaatatttgacctcaaaactaatggtgagttttgctgctttcgcagtacaaagatcttgcccagtgctgcgcctttcttctcaggcaaacccacccgtgacccgtggggctcacctgttgccacagaatggaagccaaaaccatacaccactacatcagggaagattatagggtgttttgctacaacttcaactgaaacccacccaggtgattgtggtctaccttacatcgatgacaatggtagagtcactggactgcacacaggatccggtggacccaaaactcccagcgcaaaattggttgtcccctatgtccatattgatatgaaaacaaaatctgttactgcccaaaagtatgacattacaaagcctgatattagttacaaaggattgatttgcaaacaattggatgaaattcggataataccaaaaggaacacgcctccacgtttctcctgcccacacagatgattatgaggaatgttcgcaccaaccagcatcactaggtagtggtgatccacgatgtccaaaatcccttactgctattgtagttgactccttaaaaccctactgtgataaggttgagggccccccccatgatgttttgcatagggttcagaaaatgctaattgatcacctctctggctttgttcctatgaatatctcttctgaaaactcaatgctctctgcatttcacaaactcaatcatgatacatcctgtggcccatacttaggtggaagaaagaaagatcatatggtaaatggtgagcctgacaaggcactgttggatttgctatcttcaaaatggaaacttgccactcaagggattgctctccctcatgagtacacaattgggctaaaagatgaattgagaccaattgagaaagttcaggaaggaaagagaaggatgatctggggttgtgatgttggggttgccacagtttgcgctgctgcatttaaaggtgttagtgacgcaataacggcaaaccaccagtatggacctgttcaagttgggattaacatggatagccccagtgttgaggcactttaccaacgaatcaagagcgctgccaaggtttttgcggtcgattactccaagtgggattcgactcaatcgcctcgggttagtgctgcctcaattgatattcttagatacttctctgatagatctccaattgttgattcagctgcaaacaccttaaaaagtcctccaatagcggtgttcaatggtgttgcagtaaaggtttcgtctggtcttccatctggtatgcctctgacttctgtaattaactctttaaatcactgcctatatgttggttgtgctatccttcaatctctggaatccaaaaacatacctgtcacttggaatctgttctcctcatttgacatgatgacttacggtgatgatggtgtttacatgttccctatcatgtttgctagtgttagtgatcaaatctttggaaaccttactgcttatggcttaaaacccacaagggtcgacaaatcagttggagctattgaaccaatcgatcctgaatctgttgttttcctaaaaagaaccatccaaaggacccctagtggcattcgaggtcttcttgatcgcagctcaatcctcagacagttctattacattaaaggtgaaaattcggatgattggaaaactcctccaaaagtcatagatcccacctccagaggtcaacagctgtggaacgcttgtctttatgctagccaacatggtgttgagttttacaataaggttctcaaattggcccagaaagctgttgaatacgaaggattacacctcgaccccccaagcttccaatcggcattggaacattacaataaccaatttagtggtgtggaggcgcggaatgaccagatcgattcgagtggcatgaccgccctacactgtgatgtgttcgaagtttgagcatgtgctcaacctgcgctaacgtgcttaaatattatgattgggacccccatttcaaattggtaatcaaccccaacaacttcctctctgttggcttttgtagtaaccctttaatgtgttgctacccagaactccttccggaatttggaactgtttgggattgcgatcggtcaccacttgaaatttacctagaatcaatacttggtgatgatgaatgggcatccacttttgacgctgttgacccagtcgttcccccaatgcactggggtgctgctggaaaaattttccagccacaccccggtgttctcatgcaccatctcattggtaaggttgctgcaggttgggaccccgatctgcctctaattcgactcgaggcggatgacgggtcaatcacagcacccgagcaaggaacaatggttggcggcgtcatcgctgaacccagcgcccagatgtcaacagctgctgatatggccaccgggaaaagcgttgattctgagtgggaggcattcttctcctttcacaccagcgtcaattggagtacatctgaaacccaaggaaagattctcttcaaacaatccttaggccctttgctcaacccatatctagaacaccttgctaagctatatgttgcgtggtctgggtcgattgaggttaggttctctatctctggctctggtgtctttggtgggaagctcgcagctattgttgtacctcctggggttgatccagtgcagagtacttcgatgctacaatacccccatgtcttgtttgatgctcgtcaggtggaaccagttatcttctctattcctgatctaagaagcaccctgtaccaccttatgtctgacactgacactacatccttggtcattatggtgtacaatgatctcatcaatccctatgccaatgatgccaactcttctgggtgtattgtcactgtcgagacaaaacctggccctgacttcaagtttcacctccttaagccacccggatctatgctaacccatggttctgtcccttctgatttaattcccaaaacatcttcgctctggatcggtaaccgctactggtcagacataactgattttgtgattcggccgtttgtcttccaagcaaatcgtcattttgactttaatcaagagaccgcagggtggagcacaccacggtttcggcctatatctgttaccattactgaacagaacggagcaaaattgggcattggagtggcaacagattacatagtgcctggaatccctgatggctggcctgacaccacaattcctggggagttgataccagctggcgattacgcaatcaccaatggtactggcaatgacatcaccacggctacaggatatgacactgctgatataattaagaacaataccaactttaggggcatgtacatatgtggttcgctccagcgtgcctggggtgataagaaaatttccaacactgcctttatcaccactgccaccctagatggtgacaacaacaacaagatcaatccctgtaataccatagaccagtcaaagatcgtcgtgtttcaagacaaccatgttggaaagaaagtgcaaacctcagacgatacattggccctgcttggttacactggcattggtgagcaggccatcgggtctgatagggaccgggttgtgcgcatcagcactctccctgaaactggtgctcgaggcggtaaccacccaattttctacaagaactccattaaattgggatatgtaattaggtctattgatgtctttaattcacaaatcttgcacacttccagacagttatcgctaaatcattacctactcccacctgattcttttgccgtctatagaataattgactcaaatggctcgtggtttgatattggaattgatagtgatgggttctcttttgttggtgtttctggctttggtaaattagaatttcccctttctgcctcctacatgggaatacaattggcaaagatccggcttgcctctaacattaggagtcccatgactaagttatgaattcaatattaggcctgattgatactgttactaacactattggtaaagctcaacagattgaattggacaaagctgcacttggtcaacagcgtgaattggctctccagcgcattggcttggaccgccaagccttaaacaaccaagttgagcagtttaacaaaattcttgagcaaagggtacaaggcccaatccaatccgttcgccttgcacgcgcggctggatttagggttgacccttactcatacacaaaccaaaacttttatgacgatcaattaaatgcaattagactatcatataaaaatttgtttaaaatttgatcatatatccctttgggctgccgcacctgcgcctaaccccaggg

SEQ ID NO: 62 - DNA, 7684 bp, Feline calicivirus
  misc_feature (5829)..(5829): n is a, c, g, or t
gtaaaagaaatttgagacaatgtctcaaactctgagcttcgtgcttaaaactcacagtgtccgaaaggactttgtgcactctgtcaagttaacacttgcacggaggcgcgatcttcagtatatttataacaagctctcacgcactatacgtgctgaggcttgcccttcttgtgctagttacgacgtatgtcctaactgcacctctggtgacgtcccggatgacgggtcttcgacaatgtcgattccatcatgggaggatgtcacaaagtcttcaacctactctctcctgctctctgaggacacctccgacgagttatgccctgaggacttggttaatgtggctgctcatatccgtaaggcgctatccactcagtcccacccggccaatgctgaaatgtgcaaagaacagctcacttccttattagtcatggctgaggcgatgctgccccaacgatcccgagcgtcaatcccactgcaccaacaacacacggctgcacggttggaatggagggagaaattcttctctaaacctcttgactttctccttgaaagagttggtgtgtcaaaagatattctccaaactactgcgatttggaaaattatcttggaaaaagcatgctattgtaaatcctatggagagcagtggttcactgctgccaagcaaaagttaagggaaatgaaaaactttgagagtgatacgctaaaacctcttattggtggatttatagatggtctacggttcttgaccgtggacaacccaaacccgatgggtttcctcccaaaactcatagggcttgtaaaacccctgaatttggcgatgattattgataatcatgaaaacacaatatctggctggatcatcacattaaccgcaataatggagctatacaacatcaccgaatgcaccatagatattataacatcagtcattacggctttctatgataaaattggcaaggcaaccaaattttacagttgtgttaaggcgctgttcactggatttagatctgaggacgtagcgaattccttttggtacatggcagcagcgattctatgttacctgatcactgggttaatcccaaacaatggcagattttcaaagataaaagcttgcctggccggagcgacaactcttgtatcaggtatagttgccacacaaaagctagctgcaatgttcgcaacatggaactctgagtccattgttaatgagttgtcagcaagaactgttgccctatcagagctaaacaatccaacaacaacgtctgacacggattcggtagaacgactgctagaattggctaagatcttgcatgaggagatcaagattcatactctaaaccccatcatgcaatcatacaatccaatcttgagaaatttaatgtcaaccttggacggtgttataacatcatgcaacaagaggaaagctattgctcggaagagacaggtgccagtttgttacatattaactggcccacctggatgtgggaagacaaccgcagctcaagcattagctaagaaattgtctgatcaagagccgtcggtaattaaccttgatgttgatcatcatgacacatatactggaaatgaggtatgtatcattgatgagtttgattcgtctgacaaggtagactatgcaaattttgtgattgggatggtaaactctgctcctatggtgttaaattgtgacatgcttgagaacaagggaaagctcttcacctcaaagtatataattatgacttccaactctgaaactccagtgaaaccctcttccaagcgcgcaggtgcattctaccgaagggttactatcatcgatgtaactaaccctttggtggagtcgcacaagcgtgcaaggcctgggacgtctgttcctcgtagctgctataagaaaaacttctcccatctctcacttgctaaacgaggggccgagtgctggtgcaaggaatacgttcttgaccctaaggggcttcaacaccaaagcatgaaggctccccctcctacctttcttaacattgactctttagctcagacgatgaagcaagacttcttgctcaagaacatggcttttgaggctgaagatgggtgcgcagaacatcgatatgggtttgtgtgtcaacaggaagaggttgaaactgttcgcaggctcctcaacgcggttagggcaaggatgaatgctaccttcactgtgtgtgttggacccgagacctcgcactcgattggttgcactgcgcacgtgttaactcccaatgagacctttaatggaaagaagtttgttgtgtcacgatgtaacgaagcatcactttctgcccttgaaggtaactgtgtaaagtcagctttgggcgtgtgtatgtcagataaggatctcactcatttatgccacttcattaaagggaaaattgtcaatgacagtgttaggttggatgaactacccgccaatcagcatgtggtaaccgttaattcggtgtttgatttggcctgggctcttcgtcgtcatctcacactggcagggcagtttcaagctatcagagccgcatatgatgtgcttactgtccccgacaagatccctgcaatgttgcgtcactggatggatgagacctccttttctgatgaccacgttgtgacacaatttgtaacacctggtggcatagtcatcctggagtcttgcggtggtgcacgcatctgggctttaggtcacaacgtgatccgagcaggaggtgtcaccgcaaccccaaccggaggatgtgttaggttaatgggattgtctgccccaaccatgccatggtccgagatctttcgtgagctcttctctctcttaggtagaatttggtcatctgtcaaagtatcagccctagtactaactgctcttggaatgtacgcatctagatttagaccaaaatcggaagcaaaaggaaaaaccaaattgaagattggaacatacaggggtcgcggtgtagcgctgactgatgacgagtacgatgagtggcgcgaacacaacgcctccagaaaattggatttgtcagtggaggatttcttaatgttgcgccatcgtgccgctctaggagccgacgacaatgatgcagtaaaattccggtcgtggtggaactccagaaccaaaatggccaatgattatgaggatgtcaccgtaattggcaaaggtggcgtcaaacatgaaaagatcagaaccaataccctaaaagctgtggatcgtggttatgacgtcagctttgctgaggaatcaggaccaggcaccaagttccacaagaatgcaattggatctgtcacagatgtttgtggggagcacaaaggctattgcatccacatgggccacggtgtttacgcatccgtagctcacgtggtgaaaggggattcatttttcttgggtgaaaggatttttgatcttaagactaatggtgaattttgctgctttcgcagcacgaagattctacctagtgctgcacctttcttttctgggaagcccactcgtgatccgtggggatcccccgtggcaactgagtggaagcctaaaatgtacacaacaacctctggaaagattctggggtgctttgcaacaacttcaactgaaactcacccgggagactgtggcctcccatatattgatgacaacgggagggtgaccggcctccacactggctctgggggacccaaaaccccaagtgccaagttggtggtgccatatgtgcatattgacatgaagactaaatccgtcactgctcaaaagtatgacgtaacaaagcctgatataagttacaaaggcttaatttgtaagcaattggatgagattaggattataccaaaaggcacacgtctccatgtctccccagcccacactgaggattatcaagaatgctcacaccaacccgcatcacttggaagcggggatccccgctgtccaaaatctctcactgctatagttgttgattctctaaaaccatactgtgagaaggttgagggtcctccacatgatgttttgcacagagttcaaaagatgcttatcgaccacctttcaggctttgtccctatgaacatttcctcggaaacctctatgctctcagctttccacaaactcaatcatgatacttcctgtggaccatacttgggtggcagaaagaaagatcacatggctaacggtgagccggacaagcagttattggatctcctgtctgcaaaatggaaattggccacccaaggcatagcactaccacatgagtacacaattgggctaaaggacgagttaaggcccgtggagaaggttagtgaagggaagagaaggatgatttggggttgtgatgttggcgtcgctactgtctgtgcagctgcgttcaagggtgttagcgatgccatcacagcaaaccaccagtacgggcctatacaggttggtatcaacatggatagccccagcgtcgaagcgctgttccaaaggatcaaaagcgcggccaaggtatttgcggtcgattattccaaatgggattcgacccaatcgcctcgtgtcagtgcagcttcaattgacatccttcgttacttctctgatcgctctccaattgttgactcagcctctaacacactgaagagccctcctgttgcaatctttaatggtgttgctgtaaaagtgtcctctggcttaccatctggaatgcctcttacctcagtaatcaattcccttaatcattgtctgtatgttgggtgtgccattcttcaatccctagaagctaaggccattcccgtcacttggaaccttttctcaacttttgatatcatgacttacggggatgatggtgtctacatgtttcctattatgtatgcaagtattagtgaccaaatttttggaaatctttcgtcctatgacctgaaaccaactcgggttgacaagtccgttggagcaattgagcctattgatcctgactctgttgttttcttgaagagaacaatcacaaggacacctcaggggataaggggtttacttgatcgcagctctataataagacaattctattatattaaaggtgagaactccgatgactggaagagccccccaaaacatattgacccaacatctcgagggcaacagctttggaatgcctgtctgtacgctagccaacatggcttggagtttttcaacaaggtttacaggctggccgagagggctgttgaatatgaagagctgcactttgaacccccaacatatgcttcggctttggatcattacaacagccagttcaatggcgtggaggcgcggtctgaccagatcgactcgagtggcatgaccgccctacactgtgatgtgttcgaagtttgagcatgtgctcaacctgcgctaacgtgcttaaatactatgattgggatccccacttcaaattggtgatcgaccctaataaatttctttctgttggattctgtgataacccgcttatgtgttgctatcctgagttgcttccagaattcggcactgtgtgggattgtgatcaatctccactgcaaatttaccttgaatctattcttggtgatgatgaatggtcttctacctatgaagccattgaccctgtcgttccaccaatgcactgggacaaaatggggaaaatcttccaacctcaccctggtatgctaatgcaccatatcatcggtgaagttgccaagggatgggatccaaacttgcctttgttccgattggaggccgatgatggatcggtgacaacccctgaacaaggaacaatggttggcggagtcattgctgaacccagcgcccaaatgtcaactgctgctgacatggcctctgggaaaagtgttgactccgaatgggaggctttcttctcattncacactagtgtaaattggagtacatctgaaacacaaggaaagattctattcaaacaatcacttggacccctgctaaacccatatcttgaacacatatctaagctttatgttgcatggtctggatctatagaggttaggttttctatttctggttctggtgtttttgggggaaaactcgctgctattgttgtgccgcctggggtagacccagtgcaaagcacatcaatgctacagtatcctcatgttctatttgatgcccgtcaggtagaacctgttatcttttcaatacctgatttgagaaacagcttgtaccatcttatgtcagatactgatactacctcccttgtaattatggtgtacaatgatcttattaatccttatgcaaatgattctaactcttctggatgtattgtcactgttgagactaaacctggaatcgatttcaagtttcaccttctgaaaccccctggatctatgcttacccatggctctatcccttcagatttaataccaaaatcttcttctctttggatagggaatcgtcactggactgacataaccgattttgtcattaggccttttgtgttccaagcaaaccgtcattttgattttaatcaggaaacagctggttggagtacgccaagattccgaccactagccgtaacggttagccaaagtaaaggagcaaaattggggaatggtattgcgaccgactacatcgtgcctgggattcctgatggatggccagacactacaatcccaacaaaactgacacccacaggcgattatgcaattacatctagtgatggtaatgacattgaaacaaaacttgaatacgaaaatgctgatgtgattaaaaacaacacaaacttcaggagcatgtacatttgtgggtcgctccaaagagcctggggtgataagaagatttctaatactggtttcataactactggtgttatctctgataattccataagcccaagcaataccattgatcaaagcaaaatcgtggtctatcaagacaatcatgtcaatagtgaagttcaaacctcagacatcacacttgcaattcttggctacactggtattggtgaggaggcaattggcgccaatcgggactcggttgtacgcataagtgtgctgccagaaacaggtgcccgtgggggaaaccatccaatcttttataagaattctatgaagcttggttacgtgatcagctccattgatgtgtttaattcccagatcttgcacacctctagacaactatcactgaataactacttactacctccagattcttttgctgtctatcgaattattgattctaatgggtcttggtttgatataggcattgattctgatggattttcttttgttggtgtctcaagttttcctaagttagagtttccactttctgcctcctatatgggaattcagttggcaaagattcgtcttgcctctaatattaggagttctatgactaaattatgaattcaatattaggcttaattgacactgttacaaatacaattggcaaagctcaacaaattgaattagataaagctgcacttggtcaacaacgcgaactggctttgcaacgaattaaccttgatcgccaggcgttgaacaaccaagttgagcaatttaacaaaattcttgagcaaagggtacaaggccccatccagtctgtgcggctcgcacgtgctgctggatttagggttgacccttactcatacacaaatcaaaatttttacgatgaccaattgaatgcaattagactatcttataggaatttgtttaaataattggccacaagtatcccttcgggctgccgcatttgcgcctaaccccaggg

SEQ ID NO: 63 - DNA, 24 bp, Feline Calicivirus
catcgatcgatgtcgacggatcca

SEQ ID NO: 64 - DNA, 25 bp, Feline Calicivirus
gtgcatccgtcgacatcgatcgatg

SEQ ID NO: 65 - DNA, 45 bp, Feline Calicivirus
tcgaggatccgccaccatggccgatgatggatcggtgacaacccc

SEQ ID NO: 66 - DNA, 46 bp, Feline Calicivirus
tcgactcgagtcataatttagtcatagaactcctaatattagaggc